European Patent Specification EP 3 500 680 B1, published October 2, 2024. Title: Double-stranded circle probes. Applicant: Olink Bioscience AB. The sequence listing filed with the application follows.

SEQUENCE LISTING (5 sequences)

SEQ ID NO: 1 - DNA, 141 bp, Artificial Sequence
  Protector strand 1
aacagctaggccagtaccaacacacacaccaaaccacaaattaacacaacaccagaagagaaagagacgacaatggttacagaacgagaaagaagaaagaagagaagcgccaggatagttgtgttaatttgcctagctgtt

SEQ ID NO: 2 - DNA, 134 bp, Artificial Sequence
  Protector strand 2
ttgtgttgagttgagtagagaggagagaagagaagaaagtaagaagcgcctggataagaagagatgcaaaagagacgacaatggttacagaacgagaaatcagaaagaactttcttctattctctcctgcgcca

SEQ ID NO: 3 - DNA, 64 bp, Artificial Sequence
  Template strand
cattgtcgctcttttgcatctctttatcctggcgcttctctctttctgatttctcgtctgtaac

SEQ ID NO: 4 - DNA, 60 bp, Artificial Sequence
  Target 1
tgggtgttgtgttaatttgtggtttggtgtgtgtgttggtactggcctagctgtttggtt

SEQ ID NO: 5 - DNA, 58 bp, Artificial Sequence
  Target 2
cttatccaggcgcttcttactttcttctcttctctcctctctactcaactcaacacaa